European Patent Specification EP 3 856 897 B1, published January 22, 2025. Title: TtGSTm34-8xHis. Applicant: Anadolu University. The sequence listing filed with the application follows.

SEQUENCE LISTING (4 sequences)

SEQ ID NO: 1 - DNA, 722 bp, Artificial Sequence
  TtGSTm34-8xHis (coding)
gtttaaacctcgagatgacaactcttggttactggggcatcagaggtttggctcaacctatccgtttcttacttgcctacttaggtgtctaatacactaataaggcctacgccaatcctgaagaatggttcggaaaggataagaatgaactcggctttgacttccccaacattccctacttaattgatggtgatcttaaacttactgaatcttctgctattcctatttatcttatcagaaagcacaaaagaaacgagttgttaggatcttctgctgacggttcttacagtgaaaaggaagttagagtcgcttaaattgttggtgttattagagatctttttaaggaactcacaggcttatgtttcaaccctgacttcaaaaacattaaagaaaagctctacactgaaaagctcgaactcttaattaagagactcggtgcttatcttggtgataaggaattcatagttggtaccttgacttatgctgattttcttttctatgaagccctcagctatattagacatatttatccccaagccatttgtgctactcttactgcttatatcaacagatttgaaaacctccctggtattaaggaatacattgctagccatgcctaagaacttaaggttttcttacctcctcaaagagctacctggtctggtccttaagacgacgacgacaaacaccaccaccaccaccaccaccactgatgagggccc

SEQ ID NO: 2 - protein, 232 aa, Artificial Sequence
  TtGSTm34-8xHis (protein)
MTTLGYWGIRGLAQPIRFLLAYLGVQYTNKAYANPEEWFGKDKNELGFDFPNIPYLIDGDLKLTESSAIPIYLIRKHKRNELLGSSADGSYSEKEVRVAQIVGVIRDLFKELTGLCFNPDFKNIKEKLYTEKLELLIKRLGAYLGDKEFIVGTLTYADFLFYEALSYIRHIYPQAICATLTAYINRFENLPGIKEYIASHAQELKVFLPPQRATWSGPQDDDDKHHHHHHHH

SEQ ID NO: 3 - DNA, 660 bp, Artificial Sequence
  TtGSTm34 (coding) [Tetrahymena thermophila] Gene ID: 7835917 |TTHERM_00661650|
atgacaactcttggttactggggcatcagaggtttggctcaacctatccgtttcttacttgcctacttaggtgtctaatacactaataaggcctacgccaatcctgaagaatggttcggaaaggataagaatgaactcggctttgacttccccaacattccctacttaattgatggtgatcttaaacttactgaatcttctgctattcctatttatcttatcagaaagcacaaaagaaacgagttgttaggatcttctgctgacggttcttacagtgaaaaggaagttagagtcgcttaaattgttggtgttattagagatctttttaaggaactcacaggcttatgtttcaaccctgacttcaaaaacattaaagaaaagctctacactgaaaagctcgaactcttaattaagagactcggtgcttatcttggtgataaggaattcatagttggtaccttgacttatgctgattttcttttctatgaagccctcagctatattagacatatttatccccaagccatttgtgctactcttactgcttatatcaacagatttgaaaacctccctggtattaaggaatacattgctagccatgcctaagaacttaaggttttcttacctcctcaaagagctacctggtctggtccttaatga

SEQ ID NO: 4 - protein, 219 aa, Artificial Sequence
  TtGSTm34 (protein) [Tetrahymena thermophila] |TTHERM_00661650|
MTTLGYWGIRGLAQPIRFLLAYLGVQYTNKAYANPEEWFGKDKNELGFDFPNIPYLIDGDLKLTESSAIPIYLIRKHKRNELLGSSADGSYSEKEVRVAQIVGVIRDLFKELTGLCFNPDFKNIKEKLYTEKLELLIKRLGAYLGDKEFIVGTLTYADFLFYEALSYIRHIYPQAICATLTAYINRFENLPGIKEYIASHAQELKVFLPPQRATWSGPQ